European Patent Specification EP 3 484 915 B1, published August 16, 2023. Title: NOVEL ANTIBODIES SPECIFICALLY BINDING TO ZIKA VIRUS EPITOPES AND USES THEREOF. Applicant: Humabs BioMed SA. The sequence listing filed with the application follows.

SEQUENCE LISTING (407 sequences)

SEQ ID NO: 1 - protein, 8 aa, Artificial Sequence
  ZKA190 CDRH1
GFTFSKYG

SEQ ID NO: 2 - protein, 8 aa, Artificial Sequence
  ZKA190 CDRH2
ISYEGSNK

SEQ ID NO: 3 - protein, 23 aa, Artificial Sequence
  ZKA190 CDRH3
AKSGTQYYDTTGYEYRGLEYFGY

SEQ ID NO: 4 - protein, 7 aa, Artificial Sequence
  ZKA190 CDRL1
QSVSSSY

SEQ ID NO: 5 - skipped

SEQ ID NO: 6 - protein, 9 aa, Artificial Sequence
  ZKA190 CDRL2 long
LIYDASSRA

SEQ ID NO: 7 - protein, 9 aa, Artificial Sequence
  ZKA190 CDRL3
QQYGRSRWT

SEQ ID NO: 8 - protein, 130 aa, Artificial Sequence
  ZKA190 VH
QVQLVESGGGVVQPGRSLRLSCAASGFTFSKYGMHWVRQAPGKGLEWVAVISYEGSNKYYADSVKGRFTISRDNSKNTLYLQMNSLRAEDTAVYYCAKSGTQYYDTTGYEYRGLEYFGYWGQGTLVTVSS

SEQ ID NO: 9 - protein, 108 aa, Artificial Sequence
  ZKA190 VL
EIVLTQSPGTLSLSPGERATLSCRASQSVSSSYLAWYQQKRGQAPRLLIYDASSRATGIPDRFSGSGSGTDFTLTISRLEPEDFAVYYCQQYGRSRWTFGQGTKVEIK

SEQ ID NO: 10 - DNA, 24 bp, Artificial Sequence
  ZKA190 CDRH1
ggattcaccttcagtaaatatggc

SEQ ID NO: 11 - DNA, 24 bp, Artificial Sequence
  ZKA190 CDRH2
atatcatatgagggaagtaataaa

SEQ ID NO: 12 - DNA, 69 bp, Artificial Sequence
  ZKA190 CDRH3
gcgaaatcggggacccaatactatgatactactggttatgagtataggggtttggaatactttggctac

SEQ ID NO: 13 - DNA, 21 bp, Artificial Sequence
  ZKA190 CDRL1
cagagtgttagtagcagttac

SEQ ID NO: 14 - skipped

SEQ ID NO: 15 - DNA, 27 bp, Artificial Sequence
  ZKA190 CDRL2 long
ctcatctatgatgcatccagcagggcc

SEQ ID NO: 16 - DNA, 27 bp, Artificial Sequence
  ZKA190 CDRL3
cagcagtatggtaggtcaaggtggaca

SEQ ID NO: 17 - DNA, 391 bp, Artificial Sequence
  ZKA190 VH
caggtgcagctggtggagtctgggggaggcgtggtccagcctgggaggtccctgagactctcctgtgcagcctctggattcaccttcagtaaatatggcatgcactgggtccgccaggctccaggcaaggggctggagtgggtggcagttatatcatatgagggaagtaataaatattatgcagactccgtgaagggccgattcaccatctccagagacaattccaagaacacgctgtatctgcaaatgaacagcctgagagctgaggacacggcagtgtattactgtgcgaaatcggggacccaatactatgatactactggttatgagtataggggtttggaatactttggctactggggccagggaaccctggtcaccgtctcctcag

SEQ ID NO: 18 - DNA, 325 bp, Artificial Sequence
  ZKA190 VL
gaaattgtgttgacgcagtctccaggcaccctgtctttgtctccaggggaaagagccaccctctcctgcagggccagtcagagtgttagtagcagttacttagcctggtaccagcagaaacgtggccaggctcccaggctcctcatctatgatgcatccagcagggccactggcatcccagacaggttcagtggcagtgggtctgggacagacttcactctcaccatcagcagactggagcctgaagattttgcagtgtattactgtcagcagtatggtaggtcaaggtggacattcggccaagggaccaaggtggaaatcaaac

SEQ ID NO: 19 - protein, 8 aa, Artificial Sequence
  ZKA185 CDRH1
GYSFTSYW

SEQ ID NO: 20 - protein, 8 aa, Artificial Sequence
  ZKA185 CDRH2
FDPSDSQT

SEQ ID NO: 21 - protein, 14 aa, Artificial Sequence
  ZKA185 CDRH3
ARRYCSSSSCYVDN

SEQ ID NO: 22 - protein, 6 aa, Artificial Sequence
  ZKA185 CDRL1
ALPNKF

SEQ ID NO: 23 - skipped

SEQ ID NO: 24 - protein, 9 aa, Artificial Sequence
  ZKA185 CDRL2 long
VIYEDNKRP

SEQ ID NO: 25 - protein, 12 aa, Artificial Sequence
  ZKA185 CDRL3
YSTDSSSNPLGV

SEQ ID NO: 26 - protein, 121 aa, Artificial Sequence
  ZKA185 VH
EVQLVQSGAEVKKPGESLRISCKGSGYSFTSYWITWVRQMPGKGLEWMAKFDPSDSQTNYSPSFQGHVTISVDKSISTAYLQWSSLKASDTAMYYCARRYCSSSSCYVDNWGQGTLVTIFS

SEQ ID NO: 27 - protein, 109 aa, Artificial Sequence
  ZKA185 VL
SYELTQPPSVSVSPGQTARITCSGDALPNKFAYWYRQKSGQAPVLVIYEDNKRPSGIPERFSGSSSGTMATLTISGAQVEDEADYHCYSTDSSSNPLGVFGGGTKLTVL

SEQ ID NO: 28 - DNA, 24 bp, Artificial Sequence
  ZKA185 CDRH1
ggatatagttttaccagttactgg

SEQ ID NO: 29 - DNA, 24 bp, Artificial Sequence
  ZKA185 CDRH2
tttgatcctagtgactctcaaacc

SEQ ID NO: 30 - DNA, 42 bp, Artificial Sequence
  ZKA185 CDRH3
gcgagaagatattgtagtagtagtagttgttatgtggacaat

SEQ ID NO: 31 - DNA, 18 bp, Artificial Sequence
  ZKA185 CDRL1
gcattgccaaataaattt

SEQ ID NO: 32 - skipped

SEQ ID NO: 33 - DNA, 27 bp, Artificial Sequence
  ZKA185 CDRL2 long
gtcatctatgaggacaacaaacgaccc

SEQ ID NO: 34 - DNA, 36 bp, Artificial Sequence
  ZKA185 CDRL3
tactcaacagacagcagttctaatcccctgggagta

SEQ ID NO: 35 - DNA, 364 bp, Artificial Sequence
  ZKA185 VH
gaagtgcagctggtgcagtccggagcagaggtgaaaaagcccggggagtctctgaggatctcctgtaagggttctggatatagttttaccagttactggatcacctgggtgcgccagatgcccgggaaaggcctggagtggatggcgaagtttgatcctagtgactctcaaaccaactacagcccgtccttccaaggccacgtcaccatctcagttgacaagtccatcagcactgcctacttgcagtggagcagcctgaaggcctcggacaccgccatgtattactgtgcgagaagatattgtagtagtagtagttgttatgtggacaattggggccagggaaccctggtcaccatcttctcag

SEQ ID NO: 36 - DNA, 328 bp, Artificial Sequence
  ZKA185 VL
tcctatgagctgacacagccaccctcggtgtcagtgtccccaggacaaacggccaggatcacctgctctggagatgcattgccaaataaatttgcttattggtaccggcagaagtcaggccaggcccctgttctggtcatctatgaggacaacaaacgaccctccgggatccctgagagattctctggctccagctcagggacaatggccaccttgactatcagtggggcccaggtggaggatgaagctgactaccactgttactcaacagacagcagttctaatcccctgggagtattcggcggagggaccaagctgaccgtcctag

SEQ ID NO: 37 - protein, 8 aa, Artificial Sequence
  ZKA230 CDRH1
GGSISSDY

SEQ ID NO: 38 - protein, 7 aa, Artificial Sequence
  ZKA230 CDRH2
IYYSGST

SEQ ID NO: 39 - protein, 17 aa, Artificial Sequence
  ZKA230 CDRH3
ARRRKYDSLWGSFAFDI

SEQ ID NO: 40 - protein, 8 aa, Artificial Sequence
  ZKA230 CDRL1
SSNIGGNY

SEQ ID NO: 41 - skipped

SEQ ID NO: 42 - protein, 9 aa, Artificial Sequence
  ZKA230 CDRL2 long
LICINDHRP

SEQ ID NO: 43 - protein, 11 aa, Artificial Sequence
  ZKA230 CDRL3
ATWDDSLGGLV

SEQ ID NO: 44 - protein, 123 aa, Artificial Sequence
  ZKA230 VH
QVQLQESGPGLVKPSETLSLTCAVSGGSISSDYWSWIRQPPGKGLEWIGYIYYSGSTNYNPSLKSRVTISVDTSKNHFSLKLNSVTAADTAVYYCARRRKYDSLWGSFAFDIWGQGTMVTVSS

SEQ ID NO: 45 - protein, 110 aa, Artificial Sequence
  ZKA230 VL
QSVLTQPPSASGTPGQRVTISCSGSSSNIGGNYVYWYQQLPGTAPKLLICINDHRPSGVPDRFSGSKSGTSASLAISGLQSEDEADYYCATWDDSLGGLVFGGGTKLTVL

SEQ ID NO: 46 - DNA, 24 bp, Artificial Sequence
  ZKA230 CDRH1
ggtggctccatcagtagtgactac

SEQ ID NO: 47 - DNA, 21 bp, Artificial Sequence
  ZKA230 CDRH2
atctattacagtgggagcacc

SEQ ID NO: 48 - DNA, 51 bp, Artificial Sequence
  ZKA230 CDRH3
gcgaggaggaggaagtatgattccctttgggggagttttgcttttgatatc

SEQ ID NO: 49 - DNA, 24 bp, Artificial Sequence
  ZKA230 CDRL1
agctccaacatcggaggtaattat

SEQ ID NO: 50 - skipped

SEQ ID NO: 51 - DNA, 27 bp, Artificial Sequence
  ZKA230 CDRL2 long
ctcatctgtattaatgatcaccggccc

SEQ ID NO: 52 - DNA, 33 bp, Artificial Sequence
  ZKA230 CDRL3
gcaacatgggatgacagcctgggtggccttgta

SEQ ID NO: 53 - DNA, 370 bp, Artificial Sequence
  ZKA230 VH
caggtgcagctgcaggagtcgggcccaggcctggtgaagccttcggagaccctgtccctcacctgcgcagtctctggtggctccatcagtagtgactactggagctggatccggcagcccccagggaagggactggagtggattgggtatatctattacagtgggagcaccaactacaacccctccctcaagagtcgagtcaccatatcagtagacacgtccaagaaccacttctccctgaagctgaactctgtgaccgctgcggacacggccgtgtattactgtgcgaggaggaggaagtatgattccctttgggggagttttgcttttgatatctggggccaagggacaatggtcaccgtctcttcag

SEQ ID NO: 54 - DNA, 331 bp, Artificial Sequence
  ZKA230 VL
cagtctgtgctgactcagccaccctcagcgtctgggacccccgggcagagggtcaccatctcttgttctggaagcagctccaacatcggaggtaattatgtatactggtaccagcagctcccaggaacggcccccaaactcctcatctgtattaatgatcaccggccctcaggggtccctgaccgattctctggctccaagtctggcacctcagcctccctggccatcagtgggctccagtccgaggatgaggctgattattactgtgcaacatgggatgacagcctgggtggccttgtattcggcggagggaccaagctgaccgtcctag

SEQ ID NO: 55 - protein, 8 aa, Artificial Sequence
  ZKA78 CDRH1
GFTFSNYA

SEQ ID NO: 56 - protein, 8 aa, Artificial Sequence
  ZKA78 CDRH2
IGRNGDSI

SEQ ID NO: 57 - protein, 16 aa, Artificial Sequence
  ZKA78 CDRH3
VKDLAIPESYRIEADY

SEQ ID NO: 58 - protein, 12 aa, Artificial Sequence
  ZKA78 CDRL1
QSVLYRSNNKNY

SEQ ID NO: 59 - skipped

SEQ ID NO: 60 - protein, 9 aa, Artificial Sequence
  ZKA78 CDRL2 long
LIYWASTRE

SEQ ID NO: 61 - protein, 9 aa, Artificial Sequence
  ZKA78 CDRL3
QQYYSSPRT

SEQ ID NO: 62 - protein, 123 aa, Artificial Sequence
  ZKA78 VH
EVQLAESGGGLVQPGGSLTLSCSGSGFTFSNYAMVWARQAPGKGLEYVSGIGRNGDSIYYTDSVKGRFTISRDNSKSMVYLQMSSLRTEDTAVYYCVKDLAIPESYRIEADYWGQGTLVIVSA

SEQ ID NO: 63 - protein, 113 aa, Artificial Sequence
  ZKA78 VL
DIVMTQSPDSLAVSLGERATINCKSSQSVLYRSNNKNYLSWYQQKPGQPPKLLIYWASTRESGVPDRFSGSGSGTDFTLTISPLQAEDVAVYYCQQYYSSPRTFGQGTKVEIK

SEQ ID NO: 64 - DNA, 24 bp, Artificial Sequence
  ZKA78 CDRH1
ggcttcacttttagtaactatgca

SEQ ID NO: 65 - DNA, 24 bp, Artificial Sequence
  ZKA78 CDRH2
atcgggcgcaacggggactctatc

SEQ ID NO: 66 - DNA, 48 bp, Artificial Sequence
  ZKA78 CDRH3
gtgaaagatctggccatccccgagtcctacagaattgaagctgattat

SEQ ID NO: 67 - DNA, 36 bp, Artificial Sequence
  ZKA78 CDRL1
cagtccgtgctgtaccgctctaacaacaagaattac

SEQ ID NO: 68 - skipped

SEQ ID NO: 69 - DNA, 27 bp, Artificial Sequence
  ZKA78 CDRL2 long
ctgatctattgggcttcaacccgggaa

SEQ ID NO: 70 - DNA, 27 bp, Artificial Sequence
  ZKA78 CDRL3
cagcagtactattctagtcctcgaact

SEQ ID NO: 71 - DNA, 370 bp, Artificial Sequence
  ZKA78 VH
gaggtgcagctggcagaatcaggcgggggactggtccagcctggcggcagcctgacactgtcttgcagtggatcaggcttcacttttagtaactatgcaatggtgtgggcaaggcaggctcctgggaagggactggagtatgtctctggcatcgggcgcaacggggactctatctactatactgatagtgtgaagggccggttcaccatcagcagagacaatagcaaatccatggtgtacctgcagatgagctccctgcgaaccgaagacacagcagtgtactattgcgtgaaagatctggccatccccgagtcctacagaattgaagctgattattggggacagggcaccctggtcatcgtgagcgccg

SEQ ID NO: 72 - DNA, 340 bp, Artificial Sequence
  ZKA78 VL
gacatcgtgatgacacagtctccagatagtctggcagtcagtctgggggagagggccactattaactgcaagagctcccagtccgtgctgtaccgctctaacaacaagaattacctgtcttggtatcagcagaagcccggacagccccctaaactgctgatctattgggcttcaacccgggaaagcggcgtcccagacagattctcaggcagcgggtccggaacagacttcaccctgacaattagccccctgcaggcagaggacgtggctgtctactattgtcagcagtactattctagtcctcgaactttcggccaggggaccaaggtggaaatcaaac

SEQ ID NO: 73 - protein, 8 aa, Artificial Sequence
  ZKA64 CDRH1
GYTFTGYH

SEQ ID NO: 74 - protein, 8 aa, Artificial Sequence
  ZKA64 CDRH2
INPNSGGT

SEQ ID NO: 75 - protein, 12 aa, Artificial Sequence
  ZKA64 CDRH3
ARMSSSIWGFDH

SEQ ID NO: 76 - protein, 6 aa, Artificial Sequence
  ZKA64 CDRL1
QSVLIN

SEQ ID NO: 77 - skipped

SEQ ID NO: 78 - protein, 9 aa, Artificial Sequence
  ZKA64 CDRL2 long
LIYGASSRA

SEQ ID NO: 79 - protein, 10 aa, Artificial Sequence
  ZKA64 CDRL3
QQYNDWPPIT

SEQ ID NO: 80 - protein, 119 aa, Artificial Sequence
  ZKA64 VH
QVQLVQSGAEVKKPGASVKVSCKASGYTFTGYHIDWVRQARGQGLEWMGRINPNSGGTNYAQKFQGRVTMTRDTSISTAYMQLSRLRSDDSAVYYCARMSSSIWGFDHWGQGTLVTVSS

SEQ ID NO: 81 - protein, 108 aa, Artificial Sequence
  ZKA64 VL
EIVMTQSPATLSVSPGERATLSCRASQSVLINLAWYQQKPGQAPRLLIYGASSRATGIPARFSGSGSGTEFTLTISSLQSEDFAVYYCQQYNDWPPITFGQGTRLEIK

SEQ ID NO: 82 - DNA, 24 bp, Artificial Sequence
  ZKA64 CDRH1
ggctacaccttcacagggtatcac

SEQ ID NO: 83 - DNA, 24 bp, Artificial Sequence
  ZKA64 CDRH2
attaaccctaattctggcgggacc

SEQ ID NO: 84 - DNA, 36 bp, Artificial Sequence
  ZKA64 CDRH3
gctcggatgagctcctctatttggggcttcgatcat

SEQ ID NO: 85 - DNA, 18 bp, Artificial Sequence
  ZKA64 CDRL1
cagtctgtgctgattaac

SEQ ID NO: 86 - skipped

SEQ ID NO: 87 - DNA, 27 bp, Artificial Sequence
  ZKA64 CDRL2 long
ctgatctatggagcatcctccagggct

SEQ ID NO: 88 - DNA, 30 bp, Artificial Sequence
  ZKA64 CDRL3
cagcagtacaatgattggccccctatcaca

SEQ ID NO: 89 - DNA, 358 bp, Artificial Sequence
  ZKA64 VH
caggtgcagctggtccagagcggagcagaggtgaagaaacccggcgcctcagtgaaggtcagctgcaaagcttccggctacaccttcacagggtatcacatcgactgggtgaggcaggcaagaggacagggactggaatggatgggacggattaaccctaattctggcgggaccaactacgcccagaagtttcagggccgagtgactatgaccagagacaccagcatctccacagcttatatgcagctgtcccggctgagatctgacgatagtgccgtctactattgtgctcggatgagctcctctatttggggcttcgatcattgggggcagggaacactggtgactgtcagttcag

SEQ ID NO: 90 - DNA, 325 bp, Artificial Sequence
  ZKA64 VL
gagatcgtgatgactcagtctccagccaccctgtcagtcagcccaggagaacgggcaaccctgtcttgcagagcctcccagtctgtgctgattaacctggcttggtaccagcagaagccaggccaggcaccccgactgctgatctatggagcatcctccagggctaccggcattcctgcacgcttcagtggatcaggaagcggaacagagtttaccctgacaatctctagtctgcagtccgaagacttcgctgtctactattgtcagcagtacaatgattggccccctatcacatttggccaggggactagactggagatcaagc

SEQ ID NO: 91 - protein, 8 aa, Artificial Sequence
  ZKA15 CDRH1
GGFINSYY

SEQ ID NO: 92 - protein, 7 aa, Artificial Sequence
  ZKA15 CDRH2
IYKSGST

SEQ ID NO: 93 - protein, 14 aa, Artificial Sequence
  ZKA15 CDRH3
ARDPYGDYVKAFDI

SEQ ID NO: 94 - protein, 11 aa, Artificial Sequence
  ZKA15 CDRL1
QSLLHSNGYNY

SEQ ID NO: 95 - skipped

SEQ ID NO: 96 - protein, 9 aa, Artificial Sequence
  ZKA15 CDRL2 long
LIYLGSNRA

SEQ ID NO: 97 - protein, 8 aa, Artificial Sequence
  ZKA15 CDRL3
MQALQTVT

SEQ ID NO: 98 - protein, 120 aa, Artificial Sequence
  ZKA15 VH
QVQLQESGPGLVKPSETLSLTCTVSGGFINSYYWSWIRQPAGKGLEWIGRIYKSGSTNYNPSLKSRVTMSLDTSKYQFSLKLRSVTAADTAVYYCARDPYGDYVKAFDIWGQGTMVTVSS

SEQ ID NO: 99 - protein, 111 aa, Artificial Sequence
  ZKA15 VL
DIVMTQSPLSLPVTPGEPASISCRSSQSLLHSNGYNYLNWYLQKPGQSPQLLIYLGSNRASGVPDRFSGSGSGTDFTLKISRVEAEDVGVYYCMQALQTVTFGPGTKVDIK

SEQ ID NO: 100 - DNA, 24 bp, Artificial Sequence
  ZKA15 CDRH1
ggtggcttcatcaatagttactac

SEQ ID NO: 101 - DNA, 21 bp, Artificial Sequence
  ZKA15 CDRH2
atctataaaagtgggagcacc

SEQ ID NO: 102 - DNA, 42 bp, Artificial Sequence
  ZKA15 CDRH3
gcgagagatccctacggtgactacgttaaggcttttgatatt

SEQ ID NO: 103 - DNA, 33 bp, Artificial Sequence
  ZKA15 CDRL1
cagagcctcctgcatagtaatggatacaactat

SEQ ID NO: 104 - skipped

SEQ ID NO: 105 - DNA, 27 bp, Artificial Sequence
  ZKA15 CDRL2 long
ctgatctatttgggttctaatcgggcc

SEQ ID NO: 106 - DNA, 24 bp, Artificial Sequence
  ZKA15 CDRL3
atgcaagctctacaaactgtcact

SEQ ID NO: 107 - DNA, 361 bp, Artificial Sequence
  ZKA15 VH
caggtgcagctgcaggagtcggggccaggactggtgaagccttcggagaccctgtccctcacctgcactgtctccggtggcttcatcaatagttactactggagctggatccggcagcccgccgggaagggactggagtggattgggcgtatctataaaagtgggagcaccaactacaacccctccctcaagagtcgagtcaccatgtcactagacacgtccaagtaccagttctccctgaagctgaggtctgtgaccgccgctgacacggccgtgtattactgtgcgagagatccctacggtgactacgttaaggcttttgatatttggggccaagggacaatggtcaccgtctcttcag

SEQ ID NO: 108 - DNA, 334 bp, Artificial Sequence
  ZKA15 VL
gatattgtgatgactcagtctccactctccctgcccgtcacccctggagagccggcctccatctcctgcaggtctagtcagagcctcctgcatagtaatggatacaactatttgaattggtacctgcagaagccagggcagtctccacagctcctgatctatttgggttctaatcgggcctccggggtccctgacaggttcagtggcagtggatcaggcacagattttacactgaaaatcagcagagtggaggctgaggatgttggggtttattactgcatgcaagctctacaaactgtcactttcggccctgggaccaaagtggatatcaaac

SEQ ID NO: 109 - protein, 8 aa, Artificial Sequence
  ZKA25 CDRH1
GFTFRSHW

SEQ ID NO: 110 - protein, 8 aa, Artificial Sequence
  ZKA25 CDRH2
IKEDGYEK

SEQ ID NO: 111 - protein, 14 aa, Artificial Sequence
  ZKA25 CDRH3
ARDLRVYSGRGFDP

SEQ ID NO: 112 - protein, 6 aa, Artificial Sequence
  ZKA25 CDRL1
KLGDKY

SEQ ID NO: 113 - skipped

SEQ ID NO: 114 - protein, 9 aa, Artificial Sequence
  ZKA25 CDRL2 long
VIYQDSKRP

SEQ ID NO: 115 - protein, 9 aa, Artificial Sequence
  ZKA25 CDRL3
QAWDSSTVV

SEQ ID NO: 116 - protein, 121 aa, Artificial Sequence
  ZKA25 VH
EVQLVESGGGLVRPGGSLRLSCAASGFTFRSHWMSWVRQAPGKGLEWVANIKEDGYEKYYVDSVKGRFTISRDNAKNSLYLQMKSLRAEDTAVYYCARDLRVYSGRGFDPWGQGTLVTVSS

SEQ ID NO: 117 - protein, 106 aa, Artificial Sequence
  ZKA25 VL
SYELTQPPSLSVSPGQTASITCSGDKLGDKYACWYQQKPGQSPVLVIYQDSKRPSGIPARFSGSNSGNTATLTISGTQAMDEADYYCQAWDSSTVVFGGGTKLTVL

SEQ ID NO: 118 - DNA, 24 bp, Artificial Sequence
  ZKA25 CDRH1
ggattcacctttagaagtcattgg

SEQ ID NO: 119 - DNA, 24 bp, Artificial Sequence
  ZKA25 CDRH2
ataaaggaagatggatatgagaaa

SEQ ID NO: 120 - DNA, 42 bp, Artificial Sequence
  ZKA25 CDRH3
gcgagagatttgagggtatatagtgggagaggtttcgacccc

SEQ ID NO: 121 - DNA, 18 bp, Artificial Sequence
  ZKA25 CDRL1
aaattgggggataaatat

SEQ ID NO: 122 - skipped

SEQ ID NO: 123 - DNA, 27 bp, Artificial Sequence
  ZKA25 CDRL2 long
gtcatctatcaagatagcaagcggccc

SEQ ID NO: 124 - DNA, 27 bp, Artificial Sequence
  ZKA25 CDRL3
caggcgtgggacagcagcactgtggta

SEQ ID NO: 125 - DNA, 364 bp, Artificial Sequence
  ZKA25 VH
gaggtgcagttggtggagtctgggggaggcttggtccggcctggggggtccctgagactctcctgtgcagcctctggattcacctttagaagtcattggatgagttgggtccgccaggctccagggaaggggctggagtgggtggccaacataaaggaagatggatatgagaaatactatgtggactctgtgaagggccgattcaccatctccagagacaacgccaagaactcactgtatctgcaaatgaagagcctgagagccgaggacacggccgtgtattactgtgcgagagatttgagggtatatagtgggagaggtttcgacccctggggccagggaaccctggtcaccgtctcctcag

SEQ ID NO: 126 - DNA, 319 bp, Artificial Sequence
  ZKA25 VL
tcctatgagctgactcagccaccctcactgtccgtgtccccaggacagacagccagcatcacctgctctggagataaattgggggataaatatgcttgctggtatcagcagaagccaggccagtcccctgtgttggtcatctatcaagatagcaagcggccctcagggatccctgcgcgattctctggctccaactctgggaacacagccactctgaccatcagcgggacccaggctatggatgaggctgactattactgtcaggcgtgggacagcagcactgtggtattcggtggagggaccaagctgaccgtcctag

SEQ ID NO: 127 - protein, 10 aa, Artificial Sequence
  ZKA35 CDRH1
GGSISTGGYY

SEQ ID NO: 128 - protein, 7 aa, Artificial Sequence
  ZKA35 CDRH2
IYYSGNT

SEQ ID NO: 129 - protein, 12 aa, Artificial Sequence
  ZKA35 CDRH3
AKGGGRERPFDY

SEQ ID NO: 130 - protein, 8 aa, Artificial Sequence
  ZKA35 CDRL1
SSNIGRNY

SEQ ID NO: 131 - skipped

SEQ ID NO: 132 - protein, 9 aa, Artificial Sequence
  ZKA35 CDRL2 long
LIYRNNQRP

SEQ ID NO: 133 - protein, 12 aa, Artificial Sequence
  ZKA35 CDRL3
VAWDDSRSGFVV

SEQ ID NO: 134 - protein, 120 aa, Artificial Sequence
  ZKA35 VH
QVQLQESGPGLVKPSQTLSLTCTVSGGSISTGGYYWSWIRQHPGKGLEWIGYIYYSGNTYYNPSLKSRVTISVDTSKKQFSLKLSSVTAADTAVYYCAKGGGRERPFDYWGQGTLVTVSS

SEQ ID NO: 135 - protein, 111 aa, Artificial Sequence
  ZKA35 VL
QSVLTQPPSASGTPGQRVTISCSGSSSNIGRNYVDWYQQLPGTAPKLLIYRNNQRPSGVPERFSGSKSGTSASLAISGLRSEDEADYYCVAWDDSRSGFVVFGGGTKVTVL

SEQ ID NO: 136 - DNA, 30 bp, Artificial Sequence
  ZKA35 CDRH1
ggtggctccatcagcactggtggttactac

SEQ ID NO: 137 - DNA, 21 bp, Artificial Sequence
  ZKA35 CDRH2
atctattacagtgggaacacc

SEQ ID NO: 138 - DNA, 36 bp, Artificial Sequence
  ZKA35 CDRH3
gcgaaaggaggagggagggagcgaccctttgactac

SEQ ID NO: 139 - DNA, 24 bp, Artificial Sequence
  ZKA35 CDRL1
agctccaacatcggaagaaattat

SEQ ID NO: 140 - skipped

SEQ ID NO: 141 - DNA, 27 bp, Artificial Sequence
  ZKA35 CDRL2 long
ctcatctataggaataatcagcggccc

SEQ ID NO: 142 - DNA, 36 bp, Artificial Sequence
  ZKA35 CDRL3
gtagcatgggatgacagccggagtggttttgtggta

SEQ ID NO: 143 - DNA, 361 bp, Artificial Sequence
  ZKA35 VH
caggtgcagctgcaggagtcgggcccaggactggtgaagccttcacagaccctgtccctcacctgcactgtctctggtggctccatcagcactggtggttactactggagctggatccgccagcacccagggaagggcctggagtggattggttacatctattacagtgggaacacctactacaacccgtccctcaagagtcgagttaccatatcagttgacacctctaagaagcagttctccctgaagctgagctctgtgactgccgcggacacggccgtgtattactgtgcgaaaggaggagggagggagcgaccctttgactactggggccagggaaccctggtcaccgtctcctcag

SEQ ID NO: 144 - DNA, 334 bp, Artificial Sequence
  ZKA35 VL
cagtctgtgctgactcagccaccctcagcgtctgggacccccgggcagagggtcaccatctcttgttctggaagcagctccaacatcggaagaaattatgtagactggtaccagcaactcccaggaacggcccccaaactcctcatctataggaataatcagcggccctcaggggtccctgagcgattctctggctccaagtctggcacctcagcctccctggccatcagtgggctccggtccgaggatgaggctgattattactgtgtagcatgggatgacagccggagtggttttgtggtattcggcggagggaccaaggtgaccgtcctag

SEQ ID NO: 145 - protein, 330 aa, Artificial Sequence
  IgG1 CH1-CH2-CH3 aa
ASTKGPSVFPLAPSSKSTSGGTAALGCLVKDYFPEPVTVSWNSGALTSGVHTFPAVLQSSGLYSLSSVVTVPSSSLGTQTYICNVNHKPSNTKVDKRVEPKSCDKTHTCPPCPAPELLGGPSVFLFPPKPKDTLMISRTPEVTCVVVDVSHEDPEVKFNWYVDGVEVHNAKTKPREEQYNSTYRVVSVLTVLHQDWLNGKEYKCKVSNKALPAPIEKTISKAKGQPREPQVYTLPPSREEMTKNQVSLTCLVKGFYPSDIAVEWESNGQPENNYKTTPPVLDSDGSFFLYSKLTVDKSRWQQGNVFSCSVMHEALHNHYTQKSLSLSPGK

SEQ ID NO: 146 - protein, 330 aa, Artificial Sequence
  IgG1 CH1-CH2-CH3 LALA aa
ASTKGPSVFPLAPSSKSTSGGTAALGCLVKDYFPEPVTVSWNSGALTSGVHTFPAVLQSSGLYSLSSVVTVPSSSLGTQTYICNVNHKPSNTKVDKKVEPKSCDKTHTCPPCPAPEAAGGPSVFLFPPKPKDTLMISRTPEVTCVVVDVSHEDPEVKFNWYVDGVEVHNAKTKPREEQYNSTYRVVSVLTVLHQDWLNGKEYKCKVSNKALPAPIEKTISKAKGQPREPQVYTLPPSRDELTKNQVSLTCLVKGFYPSDIAVEWESNGQPENNYKTTPPVLDSDGSFFLYSKLTVDKSRWQQGNVFSCSVMHEALHNHYTQKSLSLSPGK

SEQ ID NO: 147 - protein, 107 aa, Artificial Sequence [sequence omitted]

SEQ ID NO: 148 - protein, 106 aa, Artificial Sequence
  IgG CL aa
GQPKAAPSVTLFPPSSEELQANKATLVCLISDFYPGAVTVAWKADSSPVKAGVETTTPSKQSNNKYAASSYLSLTPEQWKSHRSYSCQVTHEGSTVEKTVAPTECS

SEQ ID NO: 149 - DNA, 990 bp, Artificial Sequence
  IgG1 CH1-CH2-CH3 nucl
gcgtcgaccaagggcccatcggtcttccccctggcaccctcctccaagagcacctctgggggcacagcggccctgggctgcctggtcaaggactacttccccgaacctgtgacggtctcgtggaactcaggcgccctgaccagcggcgtgcacaccttcccggctgtcctacagtcctcaggactctactccctcagcagcgtggtgaccgtgccctccagcagcttgggcacccagacctacatctgcaacgtgaatcacaagcccagcaacaccaaggtggacaagagagttgagcccaaatcttgtgacaaaactcacacatgcccaccgtgcccagcacctgaactcctggggggaccgtcagtcttcctcttccccccaaaacccaaggacaccctcatgatctcccggacccctgaggtcacatgcgtggtggtggacgtgagccacgaagaccctgaggtcaagttcaactggtacgtggacggcgtggaggtgcataatgccaagacaaagccgcgggaggagcagtacaacagcacgtaccgtgtggtcagcgtcctcaccgtcctgcaccaggactggctgaatggcaaggagtacaagtgcaaggtctccaacaaagccctcccagcccccatcgagaaaaccatctccaaagccaaagggcagccccgagaaccacaggtgtacaccctgcccccatcccgggaggagatgaccaagaaccaggtcagcctgacctgcctggtcaaaggcttctatcccagcgacatcgccgtggagtgggagagcaatgggcagccggagaacaactacaagaccacgcctcccgtgctggactccgacggctccttcttcctctatagcaagctcaccgtggacaagagcaggtggcagcaggggaacgtcttctcatgctccgtgatgcatgaggctctgcacaaccactacacgcagaagagcctctccctgtccccgggtaaa

SEQ ID NO: 150 - DNA, 990 bp, Artificial Sequence
  IgG1 CH1-CH2-CH3 LALA nucl
gcgtcgaccaagggcccatcggtcttccccctggcaccctcctccaagagcacctctgggggcacagcggccctgggctgcctggtcaaggactacttccccgaacctgtgacggtctcgtggaactcaggcgccctgaccagcggcgtgcacaccttcccggctgtcctacagtcctcaggactctactccctcagcagcgtggtgaccgtgccctccagcagcttgggcacccagacctacatctgcaacgtgaatcacaagcccagcaacaccaaggtggacaagagagttgagcccaaatcttgtgacaaaactcacacatgcccaccgtgcccagcacctgaagccgcggggggaccgtcagtcttcctcttccccccaaaacccaaggacaccctcatgatctcccggacccctgaggtcacatgcgtggtggtggacgtgagccacgaagaccctgaggtcaagttcaactggtacgtggacggcgtggaggtgcataatgccaagacaaagccgcgggaggagcagtacaacagcacgtaccgtgtggtcagcgtcctcaccgtcctgcaccaggactggctgaatggcaaggagtacaagtgcaaggtctccaacaaagccctcccagcccccatcgagaaaaccatctccaaagccaaagggcagccccgagaaccacaggtgtacaccctgcccccatcccgggaggagatgaccaagaaccaggtcagcctgacctgcctggtcaaaggcttctatcccagcgacatcgccgtggagtgggagagcaatgggcagccggagaacaactacaagaccacgcctcccgtgctggactccgacggctccttcttcctctatagcaagctcaccgtggacaagagcaggtggcagcaggggaacgtcttctcatgctccgtgatgcatgaggctctgcacaaccactacacgcagaagagcctctccctgtccccgggtaaa

SEQ ID NO: 151 - DNA, 321 bp, Artificial Sequence
  IgG CK nucl
cgtacggtggctgcaccatctgtcttcatcttcccgccatctgatgagcagttgaaatctggaactgcctctgttgtgtgcctgctgaataacttctatcccagagaggccaaagtacagtggaaggtggataacgccctccaatcgggtaactcccaggagagtgtcacagagcaggacagcaaggacagcacctacagcctcagcagcaccctgacgctgagcaaagcagactacgagaaacacaaagtctacgcctgcgaagtcacccatcagggcctgagctcgcccgtcacaaagagcttcaacaggggagagtgt

SEQ ID NO: 152 - DNA, 318 bp, Artificial Sequence
  IgG CL nucl
ggtcagcccaaggctgccccctcggtcactctgttcccgccctcctctgaggagcttcaagccaacaaggccacactggtgtgtctcataagtgacttctacccgggagccgtgacagtggcttggaaagcagatagcagccccgtcaaggcgggagtggagaccaccacaccctccaaacaaagcaacaacaagtacgcggccagcagctatctgagcctgacgcctgagcagtggaagtcccacagaagctacagctgccaggtcacgcatgaagggagcaccgtggagaagacagtggcccctacagaatgttca

SEQ ID NO: 153 - protein, 8 aa, Artificial Sequence
  ZKA10 CDRH1
GFTFSDSY

SEQ ID NO: 154 - protein, 8 aa, Artificial Sequence
  ZKA10 CDRH2
ISSSSPFT

SEQ ID NO: 155 - protein, 17 aa, Artificial Sequence
  ZKA10 CDRH3
ARGLVRDGYKWLYFFDY

SEQ ID NO: 156 - protein, 124 aa, Artificial Sequence
  ZKA10 VH
QVQLVESGGGLVEPRGSLRLSCAASGFTFSDSYMSWIRQAPGKGLEWISYISSSSPFTNYADSVKGRFTISRDNAKNSLYLQMNSLRAEDTAVYYCARGLVRDGYKWLYFFDYWGQGTLVTVSS

SEQ ID NO: 157 - protein, 8 aa, Artificial Sequence
  ZKA18 CDRH1
GFTFSSYG

SEQ ID NO: 158 - protein, 8 aa, Artificial Sequence
  ZKA18 CDRH2
IWYDGSNK

SEQ ID NO: 159 - protein, 13 aa, Artificial Sequence
  ZKA18 CDRH3
ARDDSGYSEPFDY

SEQ ID NO: 160 - protein, 120 aa, Artificial Sequence
  ZKA18 VH
QVQLVESGGGVVQPGRSLRLSCAASGFTFSSYGMHWVRQAPGKGLEWVAVIWYDGSNKYYADSVKGRFTITRDNSKNTLYLQMNSLRPEDTAVYYCARDDSGYSEPFDYWGQGTLVTVSS

SEQ ID NO: 161 - protein, 8 aa, Artificial Sequence
  ZKA28 CDRH1
GFTVSRNY

SEQ ID NO: 162 - protein, 7 aa, Artificial Sequence
  ZKA28 CDRH2
IYSGGST

SEQ ID NO: 163 - protein, 10 aa, Artificial Sequence
  ZKA28 CDRH3
ARWINDAFDI

SEQ ID NO: 164 - protein, 116 aa, Artificial Sequence
  ZKA28 VH
EVQLVESGGGLIQPGGSLRLSCAASGFTVSRNYMSWVRQAPGKGLEWVSVIYSGGSTYYADSVKGRFTISRDNSKNTLYLQMNSLRAEDTAVYYCARWINDAFDIWGQGTMVTVSS

SEQ ID NO: 165 - protein, 8 aa, Artificial Sequence
  ZKA29 CDRH1
GFTFSRYS

SEQ ID NO: 166 - protein, 8 aa, Artificial Sequence
  ZKA29 CDRH2
ISPRSTTI

SEQ ID NO: 167 - protein, 15 aa, Artificial Sequence
  ZKA29 CDRH3
AREDCTNGVCYRVDY

SEQ ID NO: 168 - protein, 122 aa, Artificial Sequence
  ZKA29 VH
EVQLVESGGGLVQPGGSLRLSCVVSGFTFSRYSMNWVRQAPGKGLEWVSYISPRSTTIYYADSVEGRFTVSRDNAKNSLYLQLNSLRAEDTAVYYCAREDCTNGVCYRVDYWGQGTLVTVSS

SEQ ID NO: 169 - protein, 8 aa, Artificial Sequence
  ZKA33 CDRH1
GFTFSRNW

SEQ ID NO: 170 - protein, 8 aa, Artificial Sequence
  ZKA33 CDRH2
IKEDGNEK

SEQ ID NO: 171 - protein, 15 aa, Artificial Sequence
  ZKA33 CDRH3
ARPFHQGGYAYGLAY

SEQ ID NO: 172 - protein, 122 aa, Artificial Sequence
  ZKA33 VH
EVQLVESGGGLVQPGGSLRLSCAASGFTFSRNWMTWVRQAPGKGLEWVANIKEDGNEKYYVDSVKGRFTISRDNAKNSLYLQMNSLRAEDTAVYYCARPFHQGGYAYGLAYWGQGTLVTVSS

SEQ ID NO: 173 - protein, 8 aa, Artificial Sequence
  ZKA39 CDRH1
GFTFSTYS

SEQ ID NO: 174 - protein, 8 aa, Artificial Sequence
  ZKA39 CDRH2
ISPSSSTI

SEQ ID NO: 175 - protein, 15 aa, Artificial Sequence
  ZKA39 CDRH3
AREYCSGGSCYLLDY

SEQ ID NO: 176 - protein, 122 aa, Artificial Sequence
  ZKA39 VH
EVQLVESGGGLVQPGGSLRLSCAASGFTFSTYSMNWVRQAPGKGLEWVSYISPSSSTIYYPDSLKGRFTISRDNAKNSLYLQMDSLRAEDTAQYYCAREYCSGGSCYLLDYWGQGTLVTVSS

SEQ ID NO: 177 - protein, 8 aa, Artificial Sequence
  ZKA43 CDRH1
GGSITSYY

SEQ ID NO: 178 - protein, 7 aa, Artificial Sequence
  ZKA43 CDRH2
SHYSGST

SEQ ID NO: 179 - protein, 13 aa, Artificial Sequence
  ZKA43 CDRH3
ARGIYSGKNWFDP

SEQ ID NO: 180 - protein, 119 aa, Artificial Sequence
  ZKA43 VH
QVQLQESGPGLVKPSETLSLTCTVYGGSITSYYWTWIRQPPGKGLEWIGYSHYSGSTNYNPSLKSRVTISIDTSKSQFSLNLNSVTAADTAVYYCARGIYSGKNWFDPWGQGTLVTVSS

SEQ ID NO: 181 - protein, 8 aa, Artificial Sequence
  ZKA44 CDRH1
GFTVSTSY

SEQ ID NO: 182 - protein, 7 aa, Artificial Sequence
  ZKA44 CDRH2
IYSSGST

SEQ ID NO: 183 - protein, 10 aa, Artificial Sequence
  ZKA44 CDRH3
ARVSLGGLDP

SEQ ID NO: 184 - protein, 116 aa, Artificial Sequence
  ZKA44 VH
EVQLVESGGGLIQPGGSLRLSCVASGFTVSTSYMNWVRQAPGKGLEWVSVIYSSGSTYYADSVKGRFTISRNTSKNTLYLQMNSLRAEDTAVYYCARVSLGGLDPWGQGTPVTVSS

SEQ ID NO: 185 - protein, 10 aa, Artificial Sequence
  ZKA46 CDRH1
GFSLSNGRMG

SEQ ID NO: 186 - protein, 7 aa, Artificial Sequence
  ZKA46 CDRH2
IFSNDEK

SEQ ID NO: 187 - protein, 13 aa, Artificial Sequence
  ZKA46 CDRH3
ARVEFRAGNYLDS

SEQ ID NO: 188 - protein, 121 aa, Artificial Sequence
  ZKA46 VH
QVTLKESGPVLVKPTETLTLTCTVSGFSLSNGRMGVSWIRQPPGKALEWLAHIFSNDEKYYSTSLKNRLTISKDTSKSQVVLTMTNMDPVDTATYYCARVEFRAGNYLDSWGQGTLVTVSS

SEQ ID NO: 189 - protein, 8 aa, Artificial Sequence
  ZKA50 CDRH1
GYTFTNSW

SEQ ID NO: 190 - protein, 8 aa, Artificial Sequence
  ZKA50 CDRH2
IYPGDSDT

SEQ ID NO: 191 - protein, 8 aa, Artificial Sequence
  ZKA50 CDRH3
ARQPFFDY

SEQ ID NO: 192 - protein, 115 aa, Artificial Sequence
  ZKA50 VH
EVQLVQSGAQVKKPGESLKISCKASGYTFTNSWIGWVRQMPGKGLEWMGIIYPGDSDTRYSPSFQGQVTISADKSISTAYLQWSSLKASDTAMYYCARQPFFDYWGQGTLVTVSS

SEQ ID NO: 193 - protein, 8 aa, Artificial Sequence
  ZKA54 CDRH1
GYTFTGYY

SEQ ID NO: 194 - protein, 8 aa, Artificial Sequence
  ZKA54 CDRH2
INANSGGT

SEQ ID NO: 195 - protein, 18 aa, Artificial Sequence
  ZKA54 CDRH3
AHSDIVVVPSDDYYALDV

SEQ ID NO: 196 - protein, 125 aa, Artificial Sequence
  ZKA54 VH
QVQLVQSGAEVKKPGASVKVSCKTSGYTFTGYYMHWVRQAPGQGLEWMGWINANSGGTNFAQRFQGRVTMTWDTSISTAYMELSRLRSDDTAVYYCAHSDIVVVPSDDYYALDVWGQGTTVTVSS

SEQ ID NO: 197 - protein, 8 aa, Artificial Sequence
  ZKB18 CDRH1
GYSFTSYW

SEQ ID NO: 198 - protein, 8 aa, Artificial Sequence
  ZKB18 CDRH2
IYPGDSDT

SEQ ID NO: 199 - protein, 8 aa, Artificial Sequence
  ZKB18 CDRH3
ARQTPGDY

SEQ ID NO: 200 - protein, 115 aa, Artificial Sequence
  ZKB18 VH
EVQLVQSGAEVKKPGESLKISCKTFGYSFTSYWIGWVRQMPGKGLEWMGMIYPGDSDTRYSPSFQGQVTISADMSISTAYLQWSSLKASDTAMYYCARQTPGDYWGQGTLVTVSS

SEQ ID NO: 201 - protein, 8 aa, Artificial Sequence
  ZKB20 CDRH1
GYFFTRYV

SEQ ID NO: 202 - protein, 8 aa, Artificial Sequence
  ZKB20 CDRH2
INTDNGST

SEQ ID NO: 203 - protein, 15 aa, Artificial Sequence
  ZKB20 CDRH3
ARGTGRDGYNSFFAN

SEQ ID NO: 204 - protein, 122 aa, Artificial Sequence
  ZKB20 VH
QVQLVQSGAEVKKPGASVRVSCKASGYFFTRYVILWVRQAPGQRPEWMGWINTDNGSTRYSQKFQGRVTITKDTSATTAYMDLSSLKSDDTAVYYCARGTGRDGYNSFFANWGQGTLVTVSP

SEQ ID NO: 205 - protein, 8 aa, Artificial Sequence
  ZKB21 CDRH1
GYTFTGYS

SEQ ID NO: 206 - protein, 8 aa, Artificial Sequence
  ZKB21 CDRH2
IDTNSGDT

SEQ ID NO: 207 - protein, 11 aa, Artificial Sequence
  ZKB21 CDRH3
ARDRERHPFSY

SEQ ID NO: 208 - protein, 118 aa, Artificial Sequence
  ZKB21 VH
QVQLVQSGAEVKKPGASVKVSCKASGYTFTGYSIHWVRQAPGQGLAWMGRIDTNSGDTNYAERFQGRVTMTRDTSISTAYMEVRRLRSDDTAVYYCARDRERHPFSYWGQGTLVTVSS

SEQ ID NO: 209 - protein, 10 aa, Artificial Sequence
  ZKB23 CDRH1
GGSISSGDYS

SEQ ID NO: 210 - protein, 7 aa, Artificial Sequence
  ZKB23 CDRH2
ITHSGTT

SEQ ID NO: 211 - protein, 9 aa, Artificial Sequence
  ZKB23 CDRH3
ARHFGWFDP

SEQ ID NO: 212 - protein, 117 aa, Artificial Sequence
  ZKB23 VH
QLQLQESGSGLVKPSQTLSLTCAVSGGSISSGDYSWSWIRQPPGKGLEWIGYITHSGTTYFNPSLKSRVTISVDRSRNQFSLKVTSVTAADTAVYYCARHFGWFDPWGQGTLVTVSS

SEQ ID NO: 213 - protein, 10 aa, Artificial Sequence
  ZKC29 CDRH1
GGSISSGEYF

SEQ ID NO: 214 - protein, 7 aa, Artificial Sequence
  ZKC29 CDRH2
IHNRGNT

SEQ ID NO: 215 - protein, 22 aa, Artificial Sequence
  ZKC29 CDRH3
ARGGGDLVVVPDSIWDYYGMDV

SEQ ID NO: 216 - protein, 130 aa, Artificial Sequence
  ZKC29 VH
QVQLQESGPGLVRPSQTLSLTCTVSGGSISSGEYFWTWIRQHPKKGLEWIGYIHNRGNTYYNPSLKSRLSISLDTSKNHLSLRLSSVTAADTAVYYCARGGGDLVVVPDSIWDYYGMDVWGQGTTVTVSS

SEQ ID NO: 217 - protein, 10 aa, Artificial Sequence
  ZKC31 CDRH1
GGSISSGGYH

SEQ ID NO: 218 - protein, 7 aa, Artificial Sequence
  ZKC31 CDRH2
IYYSGST

SEQ ID NO: 219 - protein, 19 aa, Artificial Sequence
  ZKC31 CDRH3
ARDRSEPGEYHYYYYAMDV

SEQ ID NO: 220 - protein, 127 aa, Artificial Sequence
  ZKC31 VH
QVQLQESGPGLVKPSQTLSLTCTVSGGSISSGGYHWSWIRQHPGKGLEWIGYIYYSGSTYYNPSLKRRVTISVDTSKNQFSLKLSSVSAADTAVYYCARDRSEPGEYHYYYYAMDVWGQGTTVTVSS

SEQ ID NO: 221 - protein, 8 aa, Artificial Sequence
  ZKC32 CDRH1
GFTVSSNY

SEQ ID NO: 222 - protein, 7 aa, Artificial Sequence
  ZKC32 CDRH2
IYSSGST

SEQ ID NO: 223 - protein, 11 aa, Artificial Sequence
  ZKC32 CDRH3
ARGKKGNAFDI

SEQ ID NO: 224 - protein, 117 aa, Artificial Sequence
  ZKC32 VH
EVQLVESGGDLIQPGGSLRLSCAASGFTVSSNYMSWVRQAPGKGLEWVSVIYSSGSTYYADSVKGRFTISRDNSKNTLYLQMNSLRAGDTAVYYCARGKKGNAFDIWGQGTVVTVSS

SEQ ID NO: 225 - protein, 10 aa, Artificial Sequence
  ZKC33, CDRH1
GDSISSRTFS

SEQ ID NO: 226 - protein, 7 aa, Artificial Sequence
  ZKC33 CDRH2
IYYSGST

SEQ ID NO: 227 - protein, 18 aa, Artificial Sequence
  ZKC33 CDRH3
ARRNAEFFSFWSYYGMDV

SEQ ID NO: 228 - protein, 126 aa, Artificial Sequence
  ZKC33 VH
QVQLQESGPGLVKPSQTLSLTCTVSGDSISSRTFSWSWIRQPPGKGLEWVGHIYYSGSTDYNPSLKSRISISIDTSKNQFSLKLSSVTAADTAVYYCARRNAEFFSFWSYYGMDVWGHGTAVIVSS

SEQ ID NO: 229 - protein, 10 aa, Artificial Sequence
  ZKC34 CDRH1
GGSINSGGYY

SEQ ID NO: 230 - protein, 7 aa, Artificial Sequence
  ZKC34 CDRH2
ILHSGNT

SEQ ID NO: 231 - protein, 15 aa, Artificial Sequence
  ZKC34 CDRH3
ARAGDYYSGYVPPEY

SEQ ID NO: 232 - protein, 123 aa, Artificial Sequence
  ZKC34 VH
QVQLQESGPGLVKPSQTLSLTCAVSGGSINSGGYYWSWVRQHPGKGLEWIGYILHSGNTNYNPSLKSRVNIFVDTSENQFSLKLRSVTAADTAIYFCARAGDYYSGYVPPEYWGPGTLVTVSS

SEQ ID NO: 233 - protein, 8 aa, Artificial Sequence
  ZKD25 CDRH1
GFTVSSNY

SEQ ID NO: 234 - protein, 7 aa, Artificial Sequence
  ZKD25 CDRH2
IYSGGST

SEQ ID NO: 235 - protein, 11 aa, Artificial Sequence
  ZKD25 CDRH3
ARFGGNPSFDY

SEQ ID NO: 236 - protein, 117 aa, Artificial Sequence
  ZKD25 VH
EVQLVESGGGLVQPGGSLRLSCAASGFTVSSNYMSWVRQAPGKGLEWVSVIYSGGSTYYANSVKGRFTISRDKSKNTLYLQMNNLRAEDTAVYFCARFGGNPSFDYWGQGTLVTVSS

SEQ ID NO: 237 - protein, 8 aa, Artificial Sequence
  ZKA3 CDRH1
GFIFSNYA

SEQ ID NO: 238 - protein, 8 aa, Artificial Sequence
  ZKA3 CDRH2
IGGKGDSI

SEQ ID NO: 239 - protein, 16 aa, Artificial Sequence
  ZKA3 CDRH3
VKDLAVLESDRLEVDQ

SEQ ID NO: 240 - protein, 123 aa, Artificial Sequence
  ZKA3 VH
EVQLAESGGGLVQPGGSLRLSCSGSGFIFSNYAMVWARQAPGKGLEYVSGIGGKGDSIYHIDSVKGRFTISRDNSKRTVYLQMSRLRTEDTAVYYCVKDLAVLESDRLEVDQWGQGTLVIVSA

SEQ ID NO: 241 - protein, 8 aa, Artificial Sequence
  ZKA4 CDRH1
GFTFSSYV

SEQ ID NO: 242 - protein, 8 aa, Artificial Sequence
  ZKA4 CDRH2
TSYDGSNK

SEQ ID NO: 243 - protein, 20 aa, Artificial Sequence
  ZKA4 CDRH3
ARGPVPYWSGESYSGAYFDF

SEQ ID NO: 244 - protein, 127 aa, Artificial Sequence
  ZKA4 VH
QVQLVESGGGVVQPGRSLRLSCAASGFTFSSYVMHWVRQAPGKGLEWVTVTSYDGSNKYYADSVKGRFTISRDNAKNTLYLQMNSLRGEDTAIYYCARGPVPYWSGESYSGAYFDFWGQGILVTVSS

SEQ ID NO: 245 - protein, 8 aa, Artificial Sequence
  ZKA5 CDRH1
GFTFSNYY

SEQ ID NO: 246 - protein, 8 aa, Artificial Sequence
  ZKA5 CDRH2
MSSSETIK

SEQ ID NO: 247 - protein, 19 aa, Artificial Sequence
  ZKA5 CDRH3
ARSGIETVAGSIDYYGMDV

SEQ ID NO: 248 - protein, 126 aa, Artificial Sequence
  ZKA5 VH
QVQLVESGGGLVKPGGSLRLSCAGSGFTFSNYYMTWIRQAPGKGLELVSYMSSSETIKYYADSVKGRFTISRDNAKNSLYLQMNSLRADDTARYYCARSGIETVAGSIDYYGMDVWGHGTPVTVSS

SEQ ID NO: 249 - protein, 8 aa, Artificial Sequence
  ZKA6 CDRH1
DFTVSNYA

SEQ ID NO: 250 - protein, 8 aa, Artificial Sequence
  ZKA6 CDRH2
VSYDGSNK

SEQ ID NO: 251 - protein, 19 aa, Artificial Sequence
  ZKA6 CDRH3
ATGVTMFQGAQTNAEYLHY

SEQ ID NO: 252 - protein, 126 aa, Artificial Sequence
  ZKA6 VH
QVHLVESGGGVVQPGRSLRLSCEASDFTVSNYAMHWVRQAPGKGLEWVAVVSYDGSNKYYADSVKGRFTISRDNSKNTLYLQMNSLRAEDTALYYCATGVTMFQGAQTNAEYLHYWGQGSLVTISS

SEQ ID NO: 253 - protein, 8 aa, Artificial Sequence
  ZKA7 CDRH1
GFTFSRYG

SEQ ID NO: 254 - protein, 8 aa, Artificial Sequence
  ZKA7 CDRH2
VSGDGSST

SEQ ID NO: 255 - protein, 15 aa, Artificial Sequence
  ZKA7 CDRH3
VKDFWSGDQSLESDF

SEQ ID NO: 256 - protein, 122 aa, Artificial Sequence
  ZKA7 VH
EVQLVESGGGLVQPGGSLRLSCSASGFTFSRYGMVWARQAPGKGLEYLSGVSGDGSSTYYANSVKGRFTISRDNSKNTLYLHMSRLRDEDTAMYYCVKDFWSGDQSLESDFWGQGALVTVSS

SEQ ID NO: 257 - protein, 8 aa, Artificial Sequence
  ZKA8 CDRH1
GFTFSAHA

SEQ ID NO: 258 - protein, 8 aa, Artificial Sequence
  ZKA8 CDRH2
ISRNEDYT

SEQ ID NO: 259 - protein, 12 aa, Artificial Sequence
  ZKA8 CDRH3
VKDFGTSPQTDF

SEQ ID NO: 260 - protein, 119 aa, Artificial Sequence
  ZKA8 VH
DERLVESGGGLVQPGGSLRLVCSASGFTFSAHAMHWVRQPPGKGLEYVSTISRNEDYTYYADSVKGRFTISRDNSKNSLYLQMRRLRPEDTAIYYCVKDFGTSPQTDFWGQGTLVAVSS

SEQ ID NO: 261 - protein, 8 aa, Artificial Sequence
  ZKA76 CDRH1
GFTFSTYF

SEQ ID NO: 262 - protein, 8 aa, Artificial Sequence
  ZKA76 CDRH2
ISSTGSYK

SEQ ID NO: 263 - protein, 17 aa, Artificial Sequence
  ZKA76 CDRH3
ARPFHSEYTYGLDAFDI

SEQ ID NO: 264 - protein, 124 aa, Artificial Sequence
  ZKA76 VH
EVQLVESGGGLVKPGGSLRLSCAASGFTFSTYFMHWVRQAPGKGLEWVASISSTGSYKFYADSVKGRFTISRDNTKNSLFLQMNSLRAEDTAVFYCARPFHSEYTYGLDAFDIWGQGTMLTVSS

SEQ ID NO: 265 - protein, 10 aa, Artificial Sequence
  ZKA117 CDRH1
GGSIRRTNSY

SEQ ID NO: 266 - protein, 7 aa, Artificial Sequence
  ZKA117 CDRH2
ISYSGST

SEQ ID NO: 267 - protein, 17 aa, Artificial Sequence
  ZKA117 CDRH3
ARLNDGSTVTTSSYFDY

SEQ ID NO: 268 - protein, 125 aa, Artificial Sequence
  ZKA117 VH
QLQLQESGPGLVKPSETLSLTCTVSGGSIRRTNSYWGWIRQTTGKGLQWIGSISYSGSTFYNPSLKSRVTISLDTSKDHFSLELSSVTAADTAIYYCARLNDGSTVTTSSYFDYWGQGTLVTVSS

SEQ ID NO: 269 - protein, 8 aa, Artificial Sequence
  ZKB27 CDRH1
GYSFTSSW

SEQ ID NO: 270 - protein, 8 aa, Artificial Sequence
  ZKB27 CDRH2
IDPSDSYT

SEQ ID NO: 271 - protein, 14 aa, Artificial Sequence
  ZKB27 CDRH3
ARHDYSVSENGMDV

SEQ ID NO: 272 - protein, 121 aa, Artificial Sequence
  ZKB27 VH
EVQLVQSGAEVKKPGESLRISCKASGYSFTSSWINWVRQMPGKGLEWMGRIDPSDSYTTYNPSFQGHVTISVDKSIGTAYLQWNSLRASDTAMYYCARHDYSVSENGMDVWGQGTTVTVSS

SEQ ID NO: 273 - protein, 8 aa, Artificial Sequence
  ZKB29 CDRH1
GFTFSSYT

SEQ ID NO: 274 - protein, 8 aa, Artificial Sequence
  ZKB29 CDRH2
ISYDGSHK

SEQ ID NO: 275 - protein, 12 aa, Artificial Sequence
  ZKB29 CDRH3
ARRSYSISCFDY

SEQ ID NO: 276 - protein, 119 aa, Artificial Sequence
  ZKB29 VH
QVQLVESGGGVVQPGRSLRLSCAASGFTFSSYTMHWVRQAPGKGLEWVAVISYDGSHKFYADSVKGRFTISRDNSKDTLYLQMNSLRAEDTALYYCARRSYSISCFDYWGQGTLVTISS

SEQ ID NO: 277 - protein, 8 aa, Artificial Sequence
  ZKB34 CDRH1
GFTFSRSG

SEQ ID NO: 278 - protein, 8 aa, Artificial Sequence
  ZKB34 CDRH2
VSYDGSNK

SEQ ID NO: 279 - protein, 19 aa, Artificial Sequence
  ZKB34 CDRH3
AKDLTMVRGVHYYYYVMDV

SEQ ID NO: 280 - protein, 126 aa, Artificial Sequence
  ZKB34 VH
QVQLVESGGGVVQPGRSLRLSCAASGFTFSRSGMHWVRQAPGKGLEWVAVVSYDGSNKYYSDSVKGRFTISRDNSKNTLYLQMNSLRVEDTAVYYCAKDLTMVRGVHYYYYVMDVWGQGTTVTVSS

SEQ ID NO: 281 - protein, 8 aa, Artificial Sequence
  ZKB39 CDRH1
GYTFDDYY

SEQ ID NO: 282 - protein, 8 aa, Artificial Sequence
  ZKB39 CDRH2
INPHRGGT

SEQ ID NO: 283 - protein, 23 aa, Artificial Sequence
  ZKB39 CDRH3
VRDQYCDGGNCYGIHQPHYGMDV

SEQ ID NO: 284 - protein, 130 aa, Artificial Sequence
  ZKB39 VH
QVQLVQSGAEVKKPGASLKVSCKASGYTFDDYYIHWVRQAPGQGLEWLGRINPHRGGTNYAQKFQGRVIMTLDMSISTTYMELRRITSDDAAVYYCVRDQYCDGGNCYGIHQPHYGMDVWGQGTTVTVSS

SEQ ID NO: 285 - protein, 8 aa, Artificial Sequence
  ZKB46 CDRH1
GYSFTSYW

SEQ ID NO: 286 - protein, 8 aa, Artificial Sequence
  ZKB46 CDRH2
IDPSDSYT

SEQ ID NO: 287 - protein, 17 aa, Artificial Sequence
  ZKB46 CDRH3
ARREYSSSSGQEDWFDP

SEQ ID NO: 288 - protein, 124 aa, Artificial Sequence
  ZKB46 VH
EVQLVQSGAEVKKPGESLRISCKGSGYSFTSYWISWVRQMPGKGLEWMGRIDPSDSYTNYSPSFQGHVTISADKSISTAYLQWSSLKASDTAMYYCARREYSSSSGQEDWFDPWGQGTLVTVSS

SEQ ID NO: 289 - protein, 8 aa, Artificial Sequence
  ZKB53 CDRH1
GFTFSSYA

SEQ ID NO: 290 - protein, 8 aa, Artificial Sequence
  ZKB53 CDRH2
ISYDGSNR

SEQ ID NO: 291 - protein, 15 aa, Artificial Sequence
  ZKB53 CDRH3
ARHVEQLPSSGYFQH

SEQ ID NO: 292 - protein, 122 aa, Artificial Sequence
  ZKB53 VH
QVQLVESGGGVVQPGRSLRLSCAASGFTFSSYAMHWVRQTPGKGLEWVTVISYDGSNRYYADSVKGRFTISRDNSKNTLYLQMNSLRSEDTAVYYCARHVEQLPSSGYFQHWGQGTLVTVSS

SEQ ID NO: 293 - protein, 8 aa, Artificial Sequence
  ZKC26 CDRH1
GFIFSDFY

SEQ ID NO: 294 - protein, 8 aa, Artificial Sequence
  ZKC26 CDRH2
IGHDGSYI

SEQ ID NO: 295 - protein, 9 aa, Artificial Sequence
  ZKC26 CDRH3
ARAHGGFRH

SEQ ID NO: 296 - protein, 116 aa, Artificial Sequence
  ZKC26 VH
QVQVVESGGGLVKPGGSLRLSCAASGFIFSDFYMSWMRQAPGKGLEWVAYIGHDGSYILYADSVKGRFTISRDNAKNSLFLRMNSLRVEDTAVYYCARAHGGFRHWGQGTVVAVSP

SEQ ID NO: 297 - protein, 8 aa, Artificial Sequence
  ZKD5 CDRH1
GFTFTSYG

SEQ ID NO: 298 - protein, 8 aa, Artificial Sequence
  ZKD5 CDRH2
ISYDGSNK

SEQ ID NO: 299 - protein, 17 aa, Artificial Sequence
  ZKD5 CDRH3
ARDRDHYDLWNAYTFDY

SEQ ID NO: 300 - protein, 124 aa, Artificial Sequence
  ZKD5 VH
QVQLVESGGGVVQPGRSLRLSCAASGFTFTSYGMHWVRQTPGKGLDWVAVISYDGSNKYYADSVKGRFTISRDNSKDTLYLQMNSLRAADTALYYCARDRDHYDLWNAYTFDYWGQGTLVTVSS

SEQ ID NO: 301 - protein, 8 aa, Artificial Sequence
  ZKD7 CDRH1
GFTFSNYA

SEQ ID NO: 302 - protein, 8 aa, Artificial Sequence
  ZKD7 CDRH2
ISYDVSDK

SEQ ID NO: 303 - protein, 20 aa, Artificial Sequence
  ZKD7 CDRH3
AGGPLGVVVIKPSNAEHFHH

SEQ ID NO: 304 - protein, 127 aa, Artificial Sequence
  ZKD7 VH
QVQLVESGGGVVQPGRSLRLSCAASGFTFSNYAMHWVRQAPGKGLEWVAVISYDVSDKYYADSVKGRFTISRDNSKNTLFLQMNSLRAEDTAAYYCAGGPLGVVVIKPSNAEHFHHWGQGTLVTVSS

SEQ ID NO: 305 - protein, 8 aa, Artificial Sequence
  ZKD8 CDRH1
GFTFINYA

SEQ ID NO: 306 - protein, 8 aa, Artificial Sequence
  ZKD8 CDRH2
ISYDGSNK

SEQ ID NO: 307 - protein, 16 aa, Artificial Sequence
  ZKD8 CDRH3
ATDADAYGDSGANFHY

SEQ ID NO: 308 - protein, 123 aa, Artificial Sequence
  ZKD8 VH
QVQLVESGGGVVQPGKSLRLSCAASGFTFINYAIHWVRQAPGKGLEWVAVISYDGSNKFYTDSVKGRFTISRDNSKNTLYLQMNSLRADDTAVYYCATDADAYGDSGANFHYWGQGTLVTVSS

SEQ ID NO: 309 - protein, 10 aa, Artificial Sequence
  ZKD15 CDRH1
DASISSGGFS

SEQ ID NO: 310 - protein, 7 aa, Artificial Sequence
  ZKD15 CDRH2
IYSSGDT

SEQ ID NO: 311 - protein, 18 aa, Artificial Sequence
  ZKD15 CDRH3
ARAHTPTSKFYYYYAMDV

SEQ ID NO: 312 - protein, 126 aa, Artificial Sequence
  ZKD15 VH
QLQLQESGSGLVKPSQTLSLTCTVSDASISSGGFSWSWIRQPLGKGLEWLGYIYSSGDTFYNPSLQGRVTMSVDIFRSQFSLKLTSVTAADTAMYYCARAHTPTSKFYYYYAMDVWGQGTTVTVSS

SEQ ID NO: 313 - protein, 8 aa, Artificial Sequence
  ZKD16 CDRH1
GFTFSDHF

SEQ ID NO: 314 - protein, 10 aa, Artificial Sequence
  ZKD16 CDRH2
SRNKPNSYTT

SEQ ID NO: 315 - protein, 17 aa, Artificial Sequence
  ZKD16 CDRH3
AKVGGCYGGDCHVENDY

SEQ ID NO: 316 - protein, 126 aa, Artificial Sequence
  ZKD16 VH
EVQLVESGGDLVQPGGSLRLSCVASGFTFSDHFMDWVRQAPGKGLEWVGRSRNKPNSYTTEYAASVKGRFSISRDDSKKALYLQMNSLQTEDTAVYYCAKVGGCYGGDCHVENDYWGQGTLVTVSS

SEQ ID NO: 317 - protein, 8 aa, Artificial Sequence
  ZKD17 CDRH1
GFIFSDYA

SEQ ID NO: 318 - protein, 8 aa, Artificial Sequence
  ZKD17 CDRH2
ISYDGSSR

SEQ ID NO: 319 - protein, 20 aa, Artificial Sequence
  ZKD17 CDRH3
ARGYCSSGTCFSTNAEYFHP

SEQ ID NO: 320 - protein, 127 aa, Artificial Sequence
  ZKD17 VH
QVQMVESGGGVVQPGTSLRLSCATSGFIFSDYAMHWVRQAPGKGLEWVAVISYDGSSRLYADSVKGRFTVSRDNSKNTLYLQMHSLRAGDTAVYYCARGYCSSGTCFSTNAEYFHPWGQGTLATISS

SEQ ID NO: 321 - protein, 8 aa, Artificial Sequence
  ZKD20 CDRH1
GFTFSDHF

SEQ ID NO: 322 - protein, 10 aa, Artificial Sequence
  ZKD20 CDRH2
SRNKPNSYTT

SEQ ID NO: 323 - protein, 17 aa, Artificial Sequence
  ZKD20 CDRH3
ARVGGCNGGDCHVENDY

SEQ ID NO: 324 - protein, 126 aa, Artificial Sequence
  ZKD20 VH
EVQLVESGGGLVQPGGSLRLSCVASGFTFSDHFMDWVRQAPGKGLEWVGRSRNKPNSYTTEYAASVKGRFTISRDDSKNSLYLQMNSLQTEDTAVYYCARVGGCNGGDCHVENDYWGQGTLVTVSS

SEQ ID NO: 325 - protein, 8 aa, Artificial Sequence
  ZKA134 CDRH1
GGTFSAYA

SEQ ID NO: 326 - protein, 8 aa, Artificial Sequence
  ZKA134 CDRH2
IIPFFGTA

SEQ ID NO: 327 - protein, 19 aa, Artificial Sequence
  ZKA134 CDRH3
ARSDIVSTTRGYHHYGMDV

SEQ ID NO: 328 - protein, 126 aa, Artificial Sequence
  ZKA134 VH
QVHLVQSGAEVKKPGSSVNVSCKASGGTFSAYAISWVRQAPGQGLEWMGGIIPFFGTAYYAQKFKGRVTVTADKSTSTVYMEMTSLRSEDTAVYYCARSDIVSTTRGYHHYGMDVWGQGTTVTVSS

SEQ ID NO: 329 - protein, 8 aa, Artificial Sequence
  ZKA246 CDRH1
GYTFSDYY

SEQ ID NO: 330 - protein, 8 aa, Artificial Sequence
  ZKA246 CDRH2
INPYSGGT

SEQ ID NO: 331 - protein, 14 aa, Artificial Sequence
  ZKA246 CDRH3
ARGFTMISDREFDP

SEQ ID NO: 332 - protein, 121 aa, Artificial Sequence
  ZKA246 VH
QVQLVQSGAEVKRPGASVKVSCKASGYTFSDYYMHWVRQAPGQGLEWMGRINPYSGGTNYAQKFHGRVTVTRDTSISTVYMELRGLRSDDTAVYYCARGFTMISDREFDPWGQGTLVTVSS

SEQ ID NO: 333 - protein, 8 aa, Artificial Sequence
  ZKA256 CDRH1
GFTFSTYW

SEQ ID NO: 334 - protein, 8 aa, Artificial Sequence
  ZKA256 CDRH2
IKQDGSEK

SEQ ID NO: 335 - protein, 20 aa, Artificial Sequence
  ZKA256 CDRH3
ARDPGYDDFWSGSYSGSFDI

SEQ ID NO: 336 - protein, 127 aa, Artificial Sequence
  ZKA256 VH
EVQLVESGGGLVQPGGSLRLSCAASGFTFSTYWMTWVRQAPGKGLEWVANIKQDGSEKYYVDSVKGRFTISRDNTKNSLYLQVNSLRAEDTAIYYCARDPGYDDFWSGSYSGSFDIWGQGTMVTVSS

SEQ ID NO: 337 - protein, 8 aa, Artificial Sequence
  ZKB42 CDRH1
GFTFNNYG

SEQ ID NO: 338 - protein, 8 aa, Artificial Sequence
  ZKB42 CDRH2
ISYDGNKK

SEQ ID NO: 339 - protein, 16 aa, Artificial Sequence
  ZKB42 CDRH3
VKYGERINGYSDPFDH

SEQ ID NO: 340 - protein, 123 aa, Artificial Sequence
  ZKB42 VH
QVQVVESGGGVVQPGRSLRLFCAASGFTFNNYGMHWVRQAPGKGLEWVALISYDGNKKYYADSVKGRFSISRDNSKNTLYLQMNRLRSGDTAVYHCVKYGERINGYSDPFDHWGQGTLVTVSS

SEQ ID NO: 341 - protein, 8 aa, Artificial Sequence
  ZKB85 CDRH1
GYTFTTYA

SEQ ID NO: 342 - protein, 8 aa, Artificial Sequence
  ZKB85 CDRH2
INTNTGNP

SEQ ID NO: 343 - protein, 11 aa, Artificial Sequence
  ZKB85 CDRH3
ARVIVPYAFDI

SEQ ID NO: 344 - protein, 118 aa, Artificial Sequence
  ZKB85 VH
QVQLVQSGSELKKPGASVKVSCKASGYTFTTYAMNWVRQAPGQGPEWVGWINTNTGNPTYAQGFTGRFVLSLDTSVSTAFLQISSLKAEDTAVYYCARVIVPYAFDIWGQGTMVTVSS

SEQ ID NO: 345 - protein, 8 aa, Artificial Sequence
  ZKB47 CDRH1
GYTFTNYY

SEQ ID NO: 346 - protein, 8 aa, Artificial Sequence
  ZKB47 CDRH2
INPSGGPT

SEQ ID NO: 347 - protein, 15 aa, Artificial Sequence
  ZKB47 CDRH3
ARDQYGGYARYGMDV

SEQ ID NO: 348 - protein, 122 aa, Artificial Sequence
  ZKB47 VH
QVQLVQSGAEVKKPGASVKVSCQASGYTFTNYYMHWVRQAPGQGLEWMGIINPSGGPTSYAQKFQGRVTMTTDTSTSTVYMELSSLRSEDTAVYYCARDQYGGYARYGMDVWGQGTTVTVSS

SEQ ID NO: 349 - protein, 8 aa, Artificial Sequence
  ZKC6 CDRH1
GYTFTGYY

SEQ ID NO: 350 - protein, 8 aa, Artificial Sequence
  ZKC6 CDRH2
INPNSGGT

SEQ ID NO: 351 - protein, 12 aa, Artificial Sequence
  ZKC6 CDRH3
ARVSDWGFAFDI

SEQ ID NO: 352 - protein, 119 aa, Artificial Sequence
  ZKC6 VH
QVQLVQSGTEVKKPGASVKVSCKASGYTFTGYYMHWVRQAPGQGLEWMGRINPNSGGTNYAQKFQGRVTMTRDTSISTAYMELSGLRSDDTAVYYCARVSDWGFAFDIWGQGTMVTVSQ

SEQ ID NO: 353 - protein, 8 aa, Artificial Sequence
  ZKA160 CDRH1
GGSITSYS

SEQ ID NO: 354 - protein, 7 aa, Artificial Sequence
  ZKA160 CDRH2
IFYSGST

SEQ ID NO: 355 - protein, 15 aa, Artificial Sequence
  ZKA160 CDRH3
ARDQTMPVWVGGMDV

SEQ ID NO: 356 - protein, 121 aa, Artificial Sequence
  ZKA160 VH
QVQLQESGPGLVKPSETLSLTCTVSGGSITSYSWSWIRQPPGKGLEWIGYIFYSGSTDYNPSLKSRVTISVDTSKDQFSLRLRSVTAADTAVYYCARDQTMPVWVGGMDVWGQGTTVTVSS

SEQ ID NO: 357 - protein, 8 aa, Artificial Sequence
  ZKA172 CDRH1
GYIFTRYW

SEQ ID NO: 358 - protein, 8 aa, Artificial Sequence
  ZKA172 CDRH2
IDPSDSYT

SEQ ID NO: 359 - protein, 13 aa, Artificial Sequence
  ZKA172 CDRH3
ARQETAREDGMAV

SEQ ID NO: 360 - protein, 120 aa, Artificial Sequence
  ZKA172 VH
EVQLVQSGAEVKKPGKSLRISCKGSGYIFTRYWISWVRQMPGKGLEWMGRIDPSDSYTNYSPSFQGHVTISADKSISTAYLQWSSLKASDTAMYYCARQETAREDGMAVWGQGTTVTVSS

SEQ ID NO: 361 - protein, 10 aa, Artificial Sequence
  ZKA174 CDRH1
GGSMSNSYYH

SEQ ID NO: 362 - protein, 7 aa, Artificial Sequence
  ZKA174 CDRH2
IYYSGST

SEQ ID NO: 363 - protein, 18 aa, Artificial Sequence
  ZKA174 CDRH3
ARNPVFNPLTLTHDAFDI

SEQ ID NO: 364 - protein, 126 aa, Artificial Sequence
  ZKA174 VH
QLQLQESGPGLVKPSETLSLTCTVSGGSMSNSYYHWGWIRQPPGKGLEWIGSIYYSGSTYYNPSLKSRVTISVDTSKNQFSLKLNSVTAADTAVYYCARNPVFNPLTLTHDAFDIWGQGTMVTVSS

SEQ ID NO: 365 - protein, 8 aa, Artificial Sequence
  ZKA189 CDRH1
GFTFSSYA

SEQ ID NO: 366 - protein, 8 aa, Artificial Sequence
  ZKA189 CDRH2
ISGSGDNT

SEQ ID NO: 367 - protein, 18 aa, Artificial Sequence
  ZKA189 CDRH3
AKWPYYDFWSGSESYFDP

SEQ ID NO: 368 - protein, 125 aa, Artificial Sequence
  ZKA189 VH
GVQLLESGGALVQPGKSLRLSCAASGFTFSSYALTWVRQAPGKGLQWVSAISGSGDNTYYADSVKGRFTISRDNSKNTLYLQMNSLRAEDTAVYYCAKWPYYDFWSGSESYFDPWGQGTLVTVSS

SEQ ID NO: 369 - protein, 8 aa, Artificial Sequence
  ZKA195 CDRH1
GYNFPSYW

SEQ ID NO: 370 - protein, 8 aa, Artificial Sequence
  ZKA195 CDRH2
IDPSDSYT

SEQ ID NO: 371 - protein, 15 aa, Artificial Sequence
  ZKA195 CDRH3
ARADCRSTSCYLVFE

SEQ ID NO: 372 - protein, 121 aa, Artificial Sequence
  ZKA195 VH
EVQLVQSGAEVKKPGESLRISCKDSGYNFPSYWIHWVRQMPGKGLEWMGTIDPSDSYTNYSPSFQGHVTISADKSISTAYLQWSSLKASDTAMYYCARADCRSTSCYLVFEGQGTLVTVSS

SEQ ID NO: 373 - protein, 8 aa, Artificial Sequence
  ZKA215 CDRH1
GYTFTSYW

SEQ ID NO: 374 - protein, 8 aa, Artificial Sequence
  ZKA215 CDRH2
IDPSDSHT

SEQ ID NO: 375 - protein, 11 aa, Artificial Sequence
  ZKA215 CDRH3
ARHALPNYFDS

SEQ ID NO: 376 - protein, 118 aa, Artificial Sequence
  ZKA215 VH
EVQLVQSGAEVKKPGESLRISCKGSGYTFTSYWISWVRQMPGKGLEWMGRIDPSDSHTDYSPSFQGHVTISADKSISAAYLQWSSLKASDTAMYYCARHALPNYFDSWGQGTLVTVSS

SEQ ID NO: 377 - protein, 8 aa, Artificial Sequence
  ZKA218 CDRH1
GFPFSSYW

SEQ ID NO: 378 - protein, 8 aa, Artificial Sequence
  ZKA218 CDRH2
INSDGRNT

SEQ ID NO: 379 - protein, 15 aa, Artificial Sequence
  ZKA218 CDRH3
ARGGYDYDSSGCFDY

SEQ ID NO: 380 - protein, 122 aa, Artificial Sequence
  ZKA218 VH
EVQLVESGGGLVQPGGSLRLSCAASGFPFSSYWMHWVRQAPGKGLVWVSRINSDGRNTNYADSVKGRFTISRDNAENTVYLQMNSLRAEDTAVYYCARGGYDYDSSGCFDYWGQGTLVTVSS

SEQ ID NO: 381 - protein, 8 aa, Artificial Sequence
  ZKB75 CDRH1
GFTFSNYA

SEQ ID NO: 382 - protein, 8 aa, Artificial Sequence
  ZKB75 CDRH2
ISGTGGST

SEQ ID NO: 383 - protein, 25 aa, Artificial Sequence
  ZKB75 CDRH3
AKDSASRGGYCSGGVCYLNPGHHDY

SEQ ID NO: 384 - protein, 132 aa, Artificial Sequence
  ZKB75 VH
EVQVLESGGGLLQPGGSLRLSCAASGFTFSNYAMSWVRQAPGKGLEWVSTISGTGGSTYYADSVKGRFTISRDNSKNTLYLQMNSLRAEDTAVYYCAKDSASRGGYCSGGVCYLNPGHHDYWGQGTLVTVSS

SEQ ID NO: 385 - protein, 8 aa, Artificial Sequence
  ZKB83 CDRH1
GYSFTNYW

SEQ ID NO: 386 - protein, 8 aa, Artificial Sequence
  ZKB83 CDRH2
IDPSDSYT

SEQ ID NO: 387 - protein, 27 aa, Artificial Sequence
  ZKB83 CDRH3
ARLRGSLYCSGGRCYSVPGETPNWFDP

SEQ ID NO: 388 - protein, 134 aa, Artificial Sequence
  ZKB83 VH
EVQLVQSGAEVKKPGESLRISCKGSGYSFTNYWITWVRQMPGKGLEWMGSIDPSDSYTNYSPSFQGHVTISADWSINTAYLQWSSLKASDTAKYYCARLRGSLYCSGGRCYSVPGETPNWFDPWGQGTLVTVSS

SEQ ID NO: 389 - protein, 8 aa, Artificial Sequence
  ZKC3 CDRH1
GGSITSYY

SEQ ID NO: 390 - protein, 7 aa, Artificial Sequence
  ZKC3 CDRH2
IYYSGST

SEQ ID NO: 391 - protein, 15 aa, Artificial Sequence
  ZKC3 CDRH3
ARVGGAPYYYYGMDV

SEQ ID NO: 392 - protein, 121 aa, Artificial Sequence
  ZKC3 VH
QVQLQESGPGLVKPSETLSLTCTVSGGSITSYYWSWIRQPPGKGLEWIGYIYYSGSTNYNPSLKSRVTISVDTSKNQFSLKLSSVTAADTAVYYCARVGGAPYYYYGMDVWGQGTTVTVSS

SEQ ID NO: 393 - protein, 8 aa, Artificial Sequence
  ZKC18 CDRH1
GFTFGDYA

SEQ ID NO: 394 - protein, 10 aa, Artificial Sequence
  ZKC18 CDRH2
IRSKAYGGTT

SEQ ID NO: 395 - protein, 13 aa, Artificial Sequence
  ZKC18 CDRH3
SRDHTGTTYAFDI

SEQ ID NO: 396 - protein, 122 aa, Artificial Sequence
  ZKC18 VH
EVQLVESGGGLVQPGRSLRLSCTASGFTFGDYAMSWFRQAPGKGLEWVGFIRSKAYGGTTEYAASVKGRFTISRDDSKSIAYLQMNSLKTEDTAVYYCSRDHTGTTYAFDIWGQGTMVTVSQ

SEQ ID NO: 397 - protein, 8 aa, Artificial Sequence
  ZKD1 CDRH1
GFTFSSYG

SEQ ID NO: 398 - protein, 8 aa, Artificial Sequence
  ZKD1 CDRH2
IWYDGSNK

SEQ ID NO: 399 - protein, 19 aa, Artificial Sequence
  ZKD1 CDRH3
ARDRRGYGDYVGYYYGMDV

SEQ ID NO: 400 - protein, 126 aa, Artificial Sequence
  ZKD1 VH
QVQLVESGGGVVQPGRSLRLSCAASGFTFSSYGMHWVRQAPGKGLEWVAVIWYDGSNKYYADSVKGRFTISRDNSKNTLYLQMNSLRAEDTAVYYCARDRRGYGDYVGYYYGMDVWGQGTTVTVSS

SEQ ID NO: 401 - protein, 95 aa, Zika virus
  misc_feature (9)..(9): Xaa can be any naturally occurring amino acid
  misc_feature (13)..(14): Xaa can be any naturally occurring amino acid
  misc_feature (22)..(22): Xaa can be any naturally occurring amino acid
  misc_feature (25)..(25): Xaa can be any naturally occurring amino acid
  misc_feature (27)..(27): Xaa can be any naturally occurring amino acid
  misc_feature (33)..(33): Xaa can be any naturally occurring amino acid
  misc_feature (35)..(35): Xaa can be any naturally occurring amino acid
  misc_feature (41)..(41): Xaa can be any naturally occurring amino acid
  misc_feature (60)..(60): Xaa can be any naturally occurring amino acid
  misc_feature (83)..(83): Xaa can be any naturally occurring amino acid
  misc_feature (85)..(85): Xaa can be any naturally occurring amino acid
TAAFTFTKXPAEXXHGTVTVEXQYXGXDGPCKXPXQMAVDXQTLTPVGRLITANPVITEXTENSKMMLELDPPFGDSYIVIGXGXKKITHHWHRS

SEQ ID NO: 402 - protein, 95 aa, Zika virus
TAAFTFTKIPAETLHGTVTVEVQYAGTDGPCKVPAQMAVDMQTLTPVGRLITANPVITESTENSKMMLELDPPFGDSYIVIGVGEKKITHHWHRS

SEQ ID NO: 403 - DNA, 20 bp, Artificial Sequence
  ZIKV-NS1 forward primer
tggagttcaactgacggtcg

SEQ ID NO: 404 - DNA, 20 bp, Artificial Sequence
  ZIKV-NS1-reverse primer
taccccgaacccatgatcct

SEQ ID NO: 405 - DNA, 21 bp, Artificial Sequence
  Gapdh- forward primer
ggcaagttcaaaggcacagtc

SEQ ID NO: 406 - DNA, 19 bp, Artificial Sequence
  Gapdh-reverse primer
caccagcatcaccccattt

SEQ ID NO: 407 - protein, 104 aa, Artificial Sequence
  ZIKV EDIII generic
  misc_feature (1)..(1): X may be any (naturally occurring) amino acid, preferably K, A, or E
  misc_feature (3)..(3): X may be any (naturally occurring) amino acid, preferably V, F, or L
  misc_feature (4)..(4): X may be any (naturally occurring) amino acid, preferably S or F
  misc_feature (17)..(17): X may be any (naturally occurring) amino acid, preferably I or V
  misc_feature (21)..(21): X may be any (naturally occurring) amino acid, preferably T or V
  misc_feature (22)..(22): X may be any (naturally occurring) amino acid, preferably L or D
  misc_feature (30)..(30): X may be any (naturally occurring) amino acid, preferably V or G
  misc_feature (33)..(33): X may be any (naturally occurring) amino acid, preferably A or G
  misc_feature (35)..(35): X may be any (naturally occurring) amino acid except R, preferably T or A
  misc_feature (41)..(41): X may be any (naturally occurring) amino acid, preferably V or I
  misc_feature (43)..(43): X may be any (naturally occurring) amino acid, preferably A or V
  misc_feature (49)..(49): X may be any (naturally occurring) amino acid, preferably M or T
  misc_feature (68)..(68): X may be any (naturally occurring) amino acid, preferably S or G
  misc_feature (70)..(70): X may be any (naturally occurring) amino acid, preferably E or K
  misc_feature (91)..(91): X may be any (naturally occurring) amino acid, preferably V or I
  misc_feature (93)..(93): X may be any (naturally occurring) amino acid, preferably E, A, K, or D
  misc_feature (94)..(94): X may be any (naturally occurring) amino acid, preferably E, A, or K, more preferably K or A
XGXXYSLCTAAFTFTKXPAEXXHGTVTVEXQYXGXDGPCKXPXQMAVDXQTLTPVGRLITANPVITEXTXNSKMMLELDPPFGDSYIVIGXGXXKITHHWHRSG